European Patent Application EP 4 759 833 A1, published June 17, 2026. Title: 抗SARS-CoV-2奥密克戎突变株XBB亚型感染的蛋白、腺病毒及疫苗. Applicant: 成都威斯克生物医药有限公司. Application CN. The sequence listing filed with the application follows.

SEQUENCE LISTING (51 sequences)

SEQ ID NO: 1 - protein, 324 aa, synthetic construct
VQPTESIVRFPNITNLCPFHEVFNATTFASVYAWNRKRISNCVADYSVIYNFAPFFAFKCYGVSPTKLNDLCFTNVYADSFVIRGNEVSQIAPGQTGNIADYNYKLPDDFTGCVIAWNSNKLDSKPSGNYNYLYRLFRKSKLKPFERDISTEIYQAGNRPCNGVAGPNCYSPLQSYGFRPTYGVGHQPYRVVVLSFELLHAPATVCGPKKSTNLVKNKSVNFNFNGLYENQKLIANQFNSAIGKIQDSLSSTASALGKLQDVVNQNAQALNTLVKQLKNHTSPDVDLGDISGINASVVNIQKEIDRLNEVAKNLNESLIDLQEL

SEQ ID NO: 2 - protein, 324 aa, synthetic construct
VQPTESIVRFPNITNLCPFHEVFNATTFASVYAWNRKRISNCVADYSVIYNFAPFFAFKCYGVSPTKLNDLCFTNVYADSFVIRGNEVSQIAPGQTGNIADYNYKLPDDFTGCVIAWNSNKLDSKPSGNYNYLYRLFRKSKLKPFERDISTEIYQAGNKPCNGVAGSNCYSPLQSYGFRPTYGVGHQPYRVVVLSFELLHAPATVCGPKKSTNLVKNKSVNFNFNGLYENQKLIANQFNSAIGKIQDSLSSTASALGKLQDVVNQNAQALNTLVKQLKNHTSPDVDLGDISGINASVVNIQKEIDRLNEVAKNLNESLIDLQEL

SEQ ID NO: 3 - protein, 226 aa, synthetic construct
VQPTESIVRFPNITNLCPFHEVFNATTFASVYAWNRKRISNCVADYSVIYNFAPFFAFKCYGVSPTKLNDLCFTNVYADSFVIRGNEVSQIAPGQTGNIADYNYKLPDDFTGCVIAWNSNKLDSKPSGNYNYLYRLFRKSKLKPFERDISTEIYQAGNKPCNGVAGPNCYSPLQSYGFRPTYGVGHQPYRVVVLSFELLHAPATVCGPKKSTNLVKNKCVNFNFNG

SEQ ID NO: 4 - protein, 226 aa, synthetic construct
VQPTESIVRFPNITNLCPFHEVFNATTFASVYAWNRKRISNCVADYSVIYNSASFSAFKCYGVSPTKLNDLCFTNVYADSFVIRGNEVSQIAPGQTGNIADYNYKLPDDFTGCVIAWNSNKLDSKPSGNYNYLYRLFRKSKLKPFERDISTEIYQAGNKPCNGVAGPNCYSPLQSYGFRPTYGVGHQPYRVVVLSFELLHAPATVCGPKKSTNLVKNKCVNFNFNG

SEQ ID NO: 5 - protein, 324 aa, synthetic construct
VQPTESIVRFPNITNLCPFHEVFNATTFASVYAWNRKRISNCVADYSVIYNFAPFFAFKCYGVSPTKLNDLCFTNVYADSFVIRGNEVSQIAPGQTGNIADYNYKLPDDFTGCVIAWNSNKLDSKPSGNYNYLYRLFRKSKLKPFERDISTEIYQAGNKPCNGVAGPNCYSPLQSYGFRPTYGVGHQPYRVVVLSFELLHAPATVCGPKKSTNLVKNKSVNFNFNGLYENQKLIANQFNSAIGKIQDSLSSTASALGKLQDVVNQNAQALNTLVKQLKNHTSPDVDLGDISGINASVVNIQKEIDRLNEVAKNLNESLIDLQEL

SEQ ID NO: 6 - protein, 324 aa, synthetic construct
VQPTESIVRFPNITNLCPFHEVFNATTFASVYAWNRKRISNCVADYSVIYNSASFSAFKCYGVSPTKLNDLCFTNVYADSFVIRGNEVSQIAPGQTGNIADYNYKLPDDFTGCVIAWNSNKLDSKPSGNYNYLYRLFRKSKLKPFERDISTEIYQAGNKPCNGVAGPNCYSPLQSYGFRPTYGVGHQPYRVVVLSFELLHAPATVCGPKKSTNLVKNKSVNFNFNGLYENQKLIANQFNSAIGKIQDSLSSTASALGKLQDVVNQNAQALNTLVKQLKNHTSPDVDLGDISGINASVVNIQKEIDRLNEVAKNLNESLIDLQEL

SEQ ID NO: 7 - protein, 226 aa, synthetic construct
VQPTESIVRFPNITNLCPFHEVFNATTFASVYAWNRKRISNCVADYSVIYNFAPFFAFKCYGVSPTKLNDLCFTNVYADSFVIRGNEVSQIAPGQTGNIADYNYKLPDDFTGCVIAWNSNKLDSKPSGNYNYLYRLFRKSKLKPFERDISTEIYQAGNKPCNGVAGPNCYSPLQSYGFRPTYGVGHQPYRVVVLSFELLHASATVCGPKKSTNLVKNKCVNFNFNG

SEQ ID NO: 8 - protein, 324 aa, synthetic construct
VQPTESIVRFPNITNLCPFHEVFNATTFASVYAWNRKRISNCVADYSVIYNFAPFFAFKCYGVSPTKLNDLCFTNVYADSFVIRGNEVSQIAPGQTGNIADYNYKLPDDFTGCVIAWNSNKLDSKPSGNYNYLYRLFRKSKLKPFERDISTEIYQAGNKPCNGVAGPNCYSPLQSYGFRPTYGVGHQPYRVVVLSFELLHASATVCGPKKSTNLVKNKSVNFNFNGLYENQKLIANQFNSAIGKIQDSLSSTASALGKLQDVVNQNAQALNTLVKQLKNHTSPDVDLGDISGINASVVNIQKEIDRLNEVAKNLNESLIDLQEL

SEQ ID NO: 9 - protein, 324 aa, synthetic construct
VQPTESIVRFPNITNLCPFHEVFNATTFASVYAWNRKRISNCVADYSVIYNFAPFFAFKCYGVSPTKLNDLCFTNVYADSFVIRGNEVSQIAPGQTGNIADYNYKLPDDFTGCVIAWNSNKLDSKPSGNYNYLYRLLRKSKLKPFERDISTEIYQAGNRPCNGVAGPNCYSPLQSYGFRPTYGVGHQPYRVVVLSFELLHAPATVCGPKKSTNLVKNKSVNFNFNGLYENQKLIANQFNSAIGKIQDSLSSTASALGKLQDVVNQNAQALNTLVKQLKNHTSPDVDLGDISGINASVVNIQKEIDRLNEVAKNLNESLIDLQEL

SEQ ID NO: 10 - protein, 323 aa, synthetic construct
VQPTESIVRFPNVTNLCPFHEVFNATRFASVYAWNRTRISNCVADYSVLYNFAPFFAFKCYGVSPTKLNDLCFTNVYADSFVIKGNEVSQIAPGQTGNIADYNYKLPDDFTGCVIAWNSNKLDSKHSGNYDYWYRLFRKSKLKPFERDISTEIYQAGNKPCKGKGPNCYFPLQSYGFRPTYGVGHQPYRVVVLSFELLHAPATVCGPKKSTNLVKNKSVNFNFNGLYENQKLIANQFNSAIGKIQDSLSSTASALGKLQDVVNQNAQALNTLVKQLKNHTSPDVDLGDISGINASVVNIQKEIDRLNEVAKNLNESLIDLQEL

SEQ ID NO: 11 - protein, 324 aa, synthetic construct
VQPTESIVRFPNITNLCPFHEVFNATTFASVYAWNRKRISNCVADYSVIYNFAPFFAFKCYGVSPTKLNDLCFTNVYADSFVIRGNEVSQIAPGQTGNIADYNYKLPDDFTGCVIAWNSNKLDSKPSGNYNYLYRLLRKSKLKPFERDISTEIYQAGNKPCNGVAGPNCYSPLQSYGFRPTYGVGHQPYRVVVLSFELLHAPATVCGPKKSTNLVKNKSVNFNFNGLYENQKLIANQFNSAIGKIQDSLSSTASALGKLQDVVNQNAQALNTLVKQLKNHTSPDVDLGDISGINASVVNIQKEIDRLNEVAKNLNESLIDLQEL

SEQ ID NO: 12 - protein, 1257 aa, synthetic construct
SQCVNLITRTQSYTNSFTRGVYYPDKVFRSSVLHSTQDLFLPFFSNVTWFHAIHVSGTNGTKRFDNPALPFNDGVYFASTEKSNIIRGWIFGTTLDSKTQSLLIVNNATNVVIKVCEFQFCNDPFLDVYQKNNKSWMESEFRVYSSANNCTFEYVSQPFLMDLVGKEGNFKNLREFVFKNIDGYFKIYSKHTPINLERDLPQGFSALEPLVDLPIGINITRFQTLLALHRSYLTPVDSSSGWTAGAAAYYVGYLQPRTFLLKYNENGTITDAVDCALDPLSETKCTLKSFTVEKGIYQTSNFRVQPTESIVRFPNITNLCPFHEVFNATTFASVYAWNRKRISNCVADYSVIYNFAPFFAFKCYGVSPTKLNDLCFTNVYADSFVIRGNEVSQIAPGQTGNIADYNYKLPDDFTGCVIAWNSNKLDSKPSGNYNYLYRLFRKSKLKPFERDISTEIYQAGNRPCNGVAGPNCYSPLQSYGFRPTYGVGHQPYRVVVLSFELLHAPATVCGPKKSTNLVKNKCVNFNFNGLTGTGVLTESNKKFLPFQQFGRDIADTTDAVRDPQTLEILDITPCSFGGVSVITPGTNTSNQVAVLYQGVNCTEVPVAIHADQLTPTWRVYSTGSNVFQTRAGCLIGAEYVNNSYECDIPIGAGICASYQTQTKSHGSASSVASQSIIAYTMSLGAENSVAYSNNSIAIPTNFTISVTTEILPVSMTKTSVDCTMYICGDSTECSNLLLQYGSFCTQLKRALTGIAVEQDKNTQEVFAQVKQIYKTPPIKYFGGFNFSQILPDPSKPSKRSPIEDLLFNKVTLADAGFIKQYGDCLGDIAARDLICAQKFNGLTVLPPLLTDEMIAQYTSALLAGTITSGWTFGAGPALQIPFPMQMAYRFNGIGVTQNVLYENQKLIANQFNSAIGKIQDSLSSTPSALGKLQDVVNHNAQALNTLVKQLSSKFGAISSVLNDILSRLDPPEAEVQIDRLITGRLQSLQTYVTQQLIRAAEIRASANLAATKMSECVLGQSKRVDFCGKGYHLMSFPQSAPHGVVFLHVTYVPAQEKNFTTAPAICHDGKAHFPREGVFVSNGTHWFVTQRNFYEPQIITTDNTFVSGNCDVVIGIVNNTVYDPLQPELDSFKEELDKYFKNHTSPDVDLGDISGINASVVNIQKEIDRLNEVAKNLNESLIDLQELGKYEQYIKWPWYIWLGFIAGLIAIVMVTIMLCCMTSCCSCLKGCCSCGSCCKFDEDDSEPVLKGVKLHYT

SEQ ID NO: 13 - protein, 1257 aa, synthetic construct
SQCVNLITRTQSYTNSFTRGVYYPDKVFRSSVLHSTQDLFLPFFSNVTWFRAIHVSGTNGTKRFDNPALPFNDGVYFASTEKSNIIRGWIFGTTLDSKTQSLLIVNNATNVVIKVCEFQFCNDPFLDVYQKNNKSWMESEFRVYSSANNCTFEYVSQPFLMDLEGKEGNFKNLREFVFKNIDGYFKIYSKHTPINLERDLPQGFSALEPLVDLPIGINITRFQTLLALHRSYLTPGGSSSGWTAGAAAYYVGYLQPRTFLLKYNENGTITDAVDCALDPLSETKCTLKSFTVEKGIYQTSNFRVQPTESIVRFPNITNLCPFHEVFNATTFASVYAWNRKRISNCVADYSVIYNFAPFFAFKCYGVSPTKLNDLCFTNVYADSFVIRGNEVSQIAPGQTGNIADYNYKLPDDFTGCVIAWNSNKLDSKPSGNYNYLYRLFRKSKLKPFERDISTEIYQAGNKPCNGVAGSNCYSPLQSYGFRPTYGVGHQPYRVVVLSFELLHAPATVCGPKKSTNLVKNKCVNFNFNGLTGTGVLTESNKKFLPFQQFGRDIADTTDAVRDPQTLEILDITPCSFGGVSVITPGTNTSNQVAVLYQGVNCTEVPVAIHADQLTPTWRVYSTGSNVFQTRAGCLIGAEYVNNSYECDIPIGAGICASYQTQTKSHGSASSVASQSIIAYTMSLGAENSVAYSNNSIAIPTNFTISVTTEILPVSMTKTSVDCTMYICGDSTECSNLLLQYGSFCTQLKRALTGIAVEQDKNTQEVFAQVKQIYKTPPIKYFGGFNFSQILPDPSKPSKRSPIEDLLFNKVTLADAGFIKQYGDCLGDIAARDLICAQKFNGLTVLPPLLTDEMIAQYTSALLAGTITSGWTFGAGPALQIPFPMQMAYRFNGIGVTQNVLYENQKLIANQFNSAIGKIQDSLSSTPSALGKLQDVVNHNAQALNTLVKQLSSKFGAISSVLNDILSRLDPPEAEVQIDRLITGRLQSLQTYVTQQLIRAAEIRASANLAATKMSECVLGQSKRVDFCGKGYHLMSFPQSAPHGVVFLHVTYVPAQEKNFTTAPAICHDGKAHFPREGVFVSNGTHWFVTQRNFYEPQIITTDNTFVSGNCDVVIGIVNNTVYDPLQPELDSFKEELDKYFKNHTSPDVDLGDISGINASVVNIQKEIDRLNEVAKNLNESLIDLQELGKYEQYIKWPWYIWLGFIAGLIAIVMVTIMLCCMTSCCSCLKGCCSCGSCCKFDEDDSEPVLKGVKLHYT

SEQ ID NO: 14 - protein, 1257 aa, synthetic construct
SQCVNLITRTQSYTNSFTRGVYYPDKVFRSSVLHSTQDLFLPFFSNVTWFHAIHVSGTNGTKRFDNPALPFNDGVYFASTEKSNIIRGWIFGTTLDSKTQSLLIVNNATNVVIKVCEFQFCNDPFLDVYQKNNKSWMESEFRVYSSANNCTFEYVSQPFLMDLEGKEGNFKNLREFVFKNIDGYFKIYSKHTPINLERDLPQGFSALEPLVDLPIGINITRFQTLLALHRSYLTPVDSSSGWTAGAAAYYVGYLQPRTFLLKYNENGTITDAVDCALDPLSETKCTLKSFTVEKGIYQTSNFRVQPTESIVRFPNITNLCPFHEVFNATTFASVYAWNRKRISNCVADYSVIYNFAPFFAFKCYGVSPTKLNDLCFTNVYADSFVIRGNEVSQIAPGQTGNIADYNYKLPDDFTGCVIAWNSNKLDSKPSGNYNYLYRLFRKSKLKPFERDISTEIYQAGNKPCNGVAGPNCYSPLQSYGFRPTYGVGHQPYRVVVLSFELLHAPATVCGPKKSTNLVKNKCVNFNFNGLTGTGVLTESNKKFLPFQQFGRDIADTTDAVRDPQTLEILDITPCSFGGVSVITPGTNTSNQVAVLYQGVNCTEVPVAIHADQLTPTWRVYSTGSNVFQTRAGCLIGAEYVNNSYECDIPIGAGICASYQTQTKSHRRARSVASQSIIAYTMSLGAENSVAYSNNSIAIPTNFTISVTTEILPVSMTKTSVDCTMYICGDSTECSNLLLQYGSFCTQLKRALTGIAVEQDKNTQEVFAQVKQIYKTPPIKYFGGFNFSQILPDPSKPSKRSFIEDLLFNKVTLADAGFIKQYGDCLGDIAARDLICAQKFNGLTVLPPLLTDEMIAQYTSALLAGTITSGWTFGAGAALQIPFAMQMAYRFNGIGVTQNVLYENQKLIANQFNSAIGKIQDSLSSTASALGKLQDVVNHNAQALNTLVKQLSSKFGAISSVLNDILSRLDKVEAEVQIDRLITGRLQSLQTYVTQQLIRAAEIRASANLAATKMSECVLGQSKRVDFCGKGYHLMSFPQSAPHGVVFLHVTYVPAQEKNFTTAPAICHDGKAHFPREGVFVSNGTHWFVTQRNFYEPQIITTDNTFVSGNCDVVIGIVNNTVYDPLQPELDSFKEELDKYFKNHTSPDVDLGDISGINASVVNIQKEIDRLNEVAKNLNESLIDLQELGKYEQYIKWPWYIWLGFIAGLIAIVMVTIMLCCMTSCCSCLKGCCSCGSCCKFDEDDSEPVLKGVKLHYT

SEQ ID NO: 15 - protein, 1257 aa, synthetic construct
SQCVNLITRTQSYTNSFTRGVYYPDKVFRSSVLHSTQDLFLPFFSNVTWFHAIHVSGTNGTKRFDNPALPFNDGVYFASTEKSNIIRGWIFGTTLDSKTQSLLIVNNATNVVIKVCEFQFCNDPFLDVYQKNNKSWMESEFRVYSSANNCTFEYVSQPFLMDLEGKEGNFKNLREFVFKNIDGYFKIYSKHTPINLERDLPQGFSALEPLVDLPIGINITRFQTLLALHRSYLTPGGSSSGWTAGAAAYYVGYLQPRTFLLKYNENGTITDAVDCALDPLSETKCTLKSFTVEKGIYQTSNFRVQPTESIVRFPNITNLCPFHEVFNATTFASVYAWNRKRISNCVADYSVIYNFAPFFAFKCYGVSPTKLNDLCFTNVYADSFVIRGNEVSQIAPGQTGNIADYNYKLPDDFTGCVIAWNSNKLDSKPSGNYNYLYRLFRKSKLKPFERDISTEIYQAGNKPCNGVAGPNCYSPLQSYGFRPTYGVGHQPYRVVVLSFELLHASATVCGPKKSTNLVKNKCVNFNFNGLTGTGVLTESNKKFLPFQQFGRDIADTTDAVRDPQTLEILDITPCSFGGVSVITPGTNTSNQVAVLYQGVNCTEVPVAIHADQLTPTWRVYSTGSNVFQTRAGCLIGAEYVNNSYECDIPIGAGICASYQTQTKSHGSASSVASQSIIAYTMSLGAENSVAYSNNSIAIPTNFTISVTTEILPVSMTKTSVDCTMYICGDSTECSNLLLQYGSFCTQLKRALTGIAVEQDKNTQEVFAQVKQIYKTPPIKYFGGFNFSQILPDPSKPSKRSPIEDLLFNKVTLADAGFIKQYGDCLGDIAARDLICAQKFNGLTVLPPLLTDEMIAQYTSALLAGTITSGWTFGAGPALQIPFPMQMAYRFNGIGVTQNVLYENQKLIANQFNSAIGKIQDSLSSTPSALGKLQDVVNHNAQALNTLVKQLSSKFGAISSVLNDILSRLDPPEAEVQIDRLITGRLQSLQTYVTQQLIRAAEIRASANLAATKMSECVLGQSKRVDFCGKGYHLMSFPQSAPHGVVFLHVTYVPAQEKNFTTAPAICHDGKAHFPREGVFVSNGTHWFVTQRNFYEPQIITTDNTFVSGNCDVVIGIVNNTVYDPLQPELDSFKEELDKYFKNHTSPDVDLGDISGINASVVNIQKEIDRLNEVAKNLNESLIDLQELGKYEQYIKWPWYIWLGFIAGLIAIVMVTIMLCCMTSCCSCLKGCCSCGSCCKFDEDDSEPVLKGVKLHYT

SEQ ID NO: 16 - protein, 492 aa, synthetic construct
MLLVNQSHQGFNKEHTSKMVSAIVLYVLLAAAAHSAFAADSIHIKDSDDLKNRLAEAGDKLVVIDFMATWCGPCKMIGPKLDEMANEMSDSIVVLKVDVDECEDIATEYNINSMPTFVFVKNSKKIEEFSGANVDKLRNTIIKLKLAGSGSGHMHHHHHHSSGDDDDKVQPTESIVRFPNITNLCPFHEVFNATTFASVYAWNRKRISNCVADYSVIYNFAPFFAFKCYGVSPTKLNDLCFTNVYADSFVIRGNEVSQIAPGQTGNIADYNYKLPDDFTGCVIAWNSNKLDSKPSGNYNYLYRLFRKSKLKPFERDISTEIYQAGNRPCNGVAGPNCYSPLQSYGFRPTYGVGHQPYRVVVLSFELLHAPATVCGPKKSTNLVKNKSVNFNFNGLYENQKLIANQFNSAIGKIQDSLSSTASALGKLQDVVNQNAQALNTLVKQLKNHTSPDVDLGDISGINASVVNIQKEIDRLNEVAKNLNESLIDLQEL

SEQ ID NO: 17 - protein, 492 aa, synthetic construct
MLLVNQSHQGFNKEHTSKMVSAIVLYVLLAAAAHSAFAADSIHIKDSDDLKNRLAEAGDKLVVIDFMATWCGPCKMIGPKLDEMANEMSDSIVVLKVDVDECEDIATEYNINSMPTFVFVKNSKKIEEFSGANVDKLRNTIIKLKLAGSGSGHMHHHHHHSSGDDDDKVQPTESIVRFPNITNLCPFHEVFNATTFASVYAWNRKRISNCVADYSVIYNFAPFFAFKCYGVSPTKLNDLCFTNVYADSFVIRGNEVSQIAPGQTGNIADYNYKLPDDFTGCVIAWNSNKLDSKPSGNYNYLYRLFRKSKLKPFERDISTEIYQAGNKPCNGVAGSNCYSPLQSYGFRPTYGVGHQPYRVVVLSFELLHAPATVCGPKKSTNLVKNKSVNFNFNGLYENQKLIANQFNSAIGKIQDSLSSTASALGKLQDVVNQNAQALNTLVKQLKNHTSPDVDLGDISGINASVVNIQKEIDRLNEVAKNLNESLIDLQEL

SEQ ID NO: 18 - protein, 394 aa, synthetic construct
MLLVNQSHQGFNKEHTSKMVSAIVLYVLLAAAAHSAFAADSIHIKDSDDLKNRLAEAGDKLVVIDFMATWCGPCKMIGPKLDEMANEMSDCIVVLKVDVDECEDIATEYNINSMPTFVFVKNSKKIEEFSGANVDKLRNTIIKLKLAGSGSGHMHHHHHHSSGDDDDKVQPTESIVRFPNITNLCPFHEVFNATTFASVYAWNRKRISNCVADYSVIYNFAPFFAFKCYGVSPTKLNDLCFTNVYADSFVIRGNEVSQIAPGQTGNIADYNYKLPDDFTGCVIAWNSNKLDSKPSGNYNYLYRLFRKSKLKPFERDISTEIYQAGNKPCNGVAGPNCYSPLQSYGFRPTYGVGHQPYRVVVLSFELLHAPATVCGPKKSTNLVKNKCVNFNFNG

SEQ ID NO: 19 - protein, 394 aa, synthetic construct
MLLVNQSHQGFNKEHTSKMVSAIVLYVLLAAAAHSAFAADSIHIKDSDDLKNRLAEAGDKLVVIDFMATWCGPCKMIGPKLDEMANEMSDCIVVLKVDVDECEDIATEYNINSMPTFVFVKNSKKIEEFSGANVDKLRNTIIKLKLAGSGSGHMHHHHHHSSGDDDDKVQPTESIVRFPNITNLCPFHEVFNATTFASVYAWNRKRISNCVADYSVIYNSASFSAFKCYGVSPTKLNDLCFTNVYADSFVIRGNEVSQIAPGQTGNIADYNYKLPDDFTGCVIAWNSNKLDSKPSGNYNYLYRLFRKSKLKPFERDISTEIYQAGNKPCNGVAGPNCYSPLQSYGFRPTYGVGHQPYRVVVLSFELLHAPATVCGPKKSTNLVKNKCVNFNFNG

SEQ ID NO: 20 - protein, 492 aa, synthetic construct
MLLVNQSHQGFNKEHTSKMVSAIVLYVLLAAAAHSAFAADSIHIKDSDDLKNRLAEAGDKLVVIDFMATWCGPCKMIGPKLDEMANEMSDSIVVLKVDVDECEDIATEYNINSMPTFVFVKNSKKIEEFSGANVDKLRNTIIKLKLAGSGSGHMHHHHHHSSGDDDDKVQPTESIVRFPNITNLCPFHEVFNATTFASVYAWNRKRISNCVADYSVIYNFAPFFAFKCYGVSPTKLNDLCFTNVYADSFVIRGNEVSQIAPGQTGNIADYNYKLPDDFTGCVIAWNSNKLDSKPSGNYNYLYRLFRKSKLKPFERDISTEIYQAGNKPCNGVAGPNCYSPLQSYGFRPTYGVGHQPYRVVVLSFELLHAPATVCGPKKSTNLVKNKSVNFNFNGLYENQKLIANQFNSAIGKIQDSLSSTASALGKLQDVVNQNAQALNTLVKQLKNHTSPDVDLGDISGINASVVNIQKEIDRLNEVAKNLNESLIDLQEL

SEQ ID NO: 21 - protein, 492 aa, synthetic construct
MLLVNQSHQGFNKEHTSKMVSAIVLYVLLAAAAHSAFAADSIHIKDSDDLKNRLAEAGDKLVVIDFMATWCGPCKMIGPKLDEMANEMSDSIVVLKVDVDECEDIATEYNINSMPTFVFVKNSKKIEEFSGANVDKLRNTIIKLKLAGSGSGHMHHHHHHSSGDDDDKVQPTESIVRFPNITNLCPFHEVFNATTFASVYAWNRKRISNCVADYSVIYNSASFSAFKCYGVSPTKLNDLCFTNVYADSFVIRGNEVSQIAPGQTGNIADYNYKLPDDFTGCVIAWNSNKLDSKPSGNYNYLYRLFRKSKLKPFERDISTEIYQAGNKPCNGVAGPNCYSPLQSYGFRPTYGVGHQPYRVVVLSFELLHAPATVCGPKKSTNLVKNKSVNFNFNGLYENQKLIANQFNSAIGKIQDSLSSTASALGKLQDVVNQNAQALNTLVKQLKNHTSPDVDLGDISGINASVVNIQKEIDRLNEVAKNLNESLIDLQEL

SEQ ID NO: 22 - protein, 394 aa, synthetic construct
MLLVNQSHQGFNKEHTSKMVSAIVLYVLLAAAAHSAFAADSIHIKDSDDLKNRLAEAGDKLVVIDFMATWCGPCKMIGPKLDEMANEMSDCIVVLKVDVDECEDIATEYNINSMPTFVFVKNSKKIEEFSGANVDKLRNTIIKLKLAGSGSGHMHHHHHHSSGDDDDKVQPTESIVRFPNITNLCPFHEVFNATTFASVYAWNRKRISNCVADYSVIYNFAPFFAFKCYGVSPTKLNDLCFTNVYADSFVIRGNEVSQIAPGQTGNIADYNYKLPDDFTGCVIAWNSNKLDSKPSGNYNYLYRLFRKSKLKPFERDISTEIYQAGNKPCNGVAGPNCYSPLQSYGFRPTYGVGHQPYRVVVLSFELLHASATVCGPKKSTNLVKNKCVNFNFNG

SEQ ID NO: 23 - protein, 492 aa, synthetic construct
MLLVNQSHQGFNKEHTSKMVSAIVLYVLLAAAAHSAFAADSIHIKDSDDLKNRLAEAGDKLVVIDFMATWCGPCKMIGPKLDEMANEMSDSIVVLKVDVDECEDIATEYNINSMPTFVFVKNSKKIEEFSGANVDKLRNTIIKLKLAGSGSGHMHHHHHHSSGDDDDKVQPTESIVRFPNITNLCPFHEVFNATTFASVYAWNRKRISNCVADYSVIYNFAPFFAFKCYGVSPTKLNDLCFTNVYADSFVIRGNEVSQIAPGQTGNIADYNYKLPDDFTGCVIAWNSNKLDSKPSGNYNYLYRLFRKSKLKPFERDISTEIYQAGNKPCNGVAGPNCYSPLQSYGFRPTYGVGHQPYRVVVLSFELLHASATVCGPKKSTNLVKNKSVNFNFNGLYENQKLIANQFNSAIGKIQDSLSSTASALGKLQDVVNQNAQALNTLVKQLKNHTSPDVDLGDISGINASVVNIQKEIDRLNEVAKNLNESLIDLQEL

SEQ ID NO: 24 - protein, 492 aa, synthetic construct
MLLVNQSHQGFNKEHTSKMVSAIVLYVLLAAAAHSAFAADSIHIKDSDDLKNRLAEAGDKLVVIDFMATWCGPCKMIGPKLDEMANEMSDSIVVLKVDVDECEDIATEYNINSMPTFVFVKNSKKIEEFSGANVDKLRNTIIKLKLAGSGSGHMHHHHHHSSGDDDDKVQPTESIVRFPNITNLCPFHEVFNATTFASVYAWNRKRISNCVADYSVIYNFAPFFAFKCYGVSPTKLNDLCFTNVYADSFVIRGNEVSQIAPGQTGNIADYNYKLPDDFTGCVIAWNSNKLDSKPSGNYNYLYRLLRKSKLKPFERDISTEIYQAGNRPCNGVAGPNCYSPLQSYGFRPTYGVGHQPYRVVVLSFELLHAPATVCGPKKSTNLVKNKSVNFNFNGLYENQKLIANQFNSAIGKIQDSLSSTASALGKLQDVVNQNAQALNTLVKQLKNHTSPDVDLGDISGINASVVNIQKEIDRLNEVAKNLNESLIDLQEL

SEQ ID NO: 25 - protein, 491 aa, synthetic construct
MLLVNQSHQGFNKEHTSKMVSAIVLYVLLAAAAHSAFAADSIHIKDSDDLKNRLAEAGDKLVVIDFMATWCGPCKMIGPKLDEMANEMSDSIVVLKVDVDECEDIATEYNINSMPTFVFVKNSKKIEEFSGANVDKLRNTIIKLKLAGSGSGHMHHHHHHSSGDDDDKVQPTESIVRFPNVTNLCPFHEVFNATRFASVYAWNRTRISNCVADYSVLYNFAPFFAFKCYGVSPTKLNDLCFTNVYADSFVIKGNEVSQIAPGQTGNIADYNYKLPDDFTGCVIAWNSNKLDSKHSGNYDYWYRLFRKSKLKPFERDISTEIYQAGNKPCKGKGPNCYFPLQSYGFRPTYGVGHQPYRVVVLSFELLHAPATVCGPKKSTNLVKNKSVNFNFNGLYENQKLIANQFNSAIGKIQDSLSSTASALGKLQDVVNQNAQALNTLVKQLKNHTSPDVDLGDISGINASVVNIQKEIDRLNEVAKNLNESLIDLQEL

SEQ ID NO: 26 - protein, 492 aa, synthetic construct
MLLVNQSHQGFNKEHTSKMVSAIVLYVLLAAAAHSAFAADSIHIKDSDDLKNRLAEAGDKLVVIDFMATWCGPCKMIGPKLDEMANEMSDSIVVLKVDVDECEDIATEYNINSMPTFVFVKNSKKIEEFSGANVDKLRNTIIKLKLAGSGSGHMHHHHHHSSGDDDDKVQPTESIVRFPNITNLCPFHEVFNATTFASVYAWNRKRISNCVADYSVIYNFAPFFAFKCYGVSPTKLNDLCFTNVYADSFVIRGNEVSQIAPGQTGNIADYNYKLPDDFTGCVIAWNSNKLDSKPSGNYNYLYRLLRKSKLKPFERDISTEIYQAGNKPCNGVAGPNCYSPLQSYGFRPTYGVGHQPYRVVVLSFELLHAPATVCGPKKSTNLVKNKSVNFNFNGLYENQKLIANQFNSAIGKIQDSLSSTASALGKLQDVVNQNAQALNTLVKQLKNHTSPDVDLGDISGINASVVNIQKEIDRLNEVAKNLNESLIDLQEL

SEQ ID NO: 27 - protein, 1269 aa, synthetic construct
MFVFLVLLPLVSSQCVNLITRTQSYTNSFTRGVYYPDKVFRSSVLHSTQDLFLPFFSNVTWFHAIHVSGTNGTKRFDNPALPFNDGVYFASTEKSNIIRGWIFGTTLDSKTQSLLIVNNATNVVIKVCEFQFCNDPFLDVYQKNNKSWMESEFRVYSSANNCTFEYVSQPFLMDLVGKEGNFKNLREFVFKNIDGYFKIYSKHTPINLERDLPQGFSALEPLVDLPIGINITRFQTLLALHRSYLTPVDSSSGWTAGAAAYYVGYLQPRTFLLKYNENGTITDAVDCALDPLSETKCTLKSFTVEKGIYQTSNFRVQPTESIVRFPNITNLCPFHEVFNATTFASVYAWNRKRISNCVADYSVIYNFAPFFAFKCYGVSPTKLNDLCFTNVYADSFVIRGNEVSQIAPGQTGNIADYNYKLPDDFTGCVIAWNSNKLDSKPSGNYNYLYRLFRKSKLKPFERDISTEIYQAGNRPCNGVAGPNCYSPLQSYGFRPTYGVGHQPYRVVVLSFELLHAPATVCGPKKSTNLVKNKCVNFNFNGLTGTGVLTESNKKFLPFQQFGRDIADTTDAVRDPQTLEILDITPCSFGGVSVITPGTNTSNQVAVLYQGVNCTEVPVAIHADQLTPTWRVYSTGSNVFQTRAGCLIGAEYVNNSYECDIPIGAGICASYQTQTKSHGSASSVASQSIIAYTMSLGAENSVAYSNNSIAIPTNFTISVTTEILPVSMTKTSVDCTMYICGDSTECSNLLLQYGSFCTQLKRALTGIAVEQDKNTQEVFAQVKQIYKTPPIKYFGGFNFSQILPDPSKPSKRSPIEDLLFNKVTLADAGFIKQYGDCLGDIAARDLICAQKFNGLTVLPPLLTDEMIAQYTSALLAGTITSGWTFGAGPALQIPFPMQMAYRFNGIGVTQNVLYENQKLIANQFNSAIGKIQDSLSSTPSALGKLQDVVNHNAQALNTLVKQLSSKFGAISSVLNDILSRLDPPEAEVQIDRLITGRLQSLQTYVTQQLIRAAEIRASANLAATKMSECVLGQSKRVDFCGKGYHLMSFPQSAPHGVVFLHVTYVPAQEKNFTTAPAICHDGKAHFPREGVFVSNGTHWFVTQRNFYEPQIITTDNTFVSGNCDVVIGIVNNTVYDPLQPELDSFKEELDKYFKNHTSPDVDLGDISGINASVVNIQKEIDRLNEVAKNLNESLIDLQELGKYEQYIKWPWYIWLGFIAGLIAIVMVTIMLCCMTSCCSCLKGCCSCGSCCKFDEDDSEPVLKGVKLHYT

SEQ ID NO: 28 - protein, 1269 aa, synthetic construct
MFVFLVLLPLVSSQCVNLITRTQSYTNSFTRGVYYPDKVFRSSVLHSTQDLFLPFFSNVTWFRAIHVSGTNGTKRFDNPALPFNDGVYFASTEKSNIIRGWIFGTTLDSKTQSLLIVNNATNVVIKVCEFQFCNDPFLDVYQKNNKSWMESEFRVYSSANNCTFEYVSQPFLMDLEGKEGNFKNLREFVFKNIDGYFKIYSKHTPINLERDLPQGFSALEPLVDLPIGINITRFQTLLALHRSYLTPGGSSSGWTAGAAAYYVGYLQPRTFLLKYNENGTITDAVDCALDPLSETKCTLKSFTVEKGIYQTSNFRVQPTESIVRFPNITNLCPFHEVFNATTFASVYAWNRKRISNCVADYSVIYNFAPFFAFKCYGVSPTKLNDLCFTNVYADSFVIRGNEVSQIAPGQTGNIADYNYKLPDDFTGCVIAWNSNKLDSKPSGNYNYLYRLFRKSKLKPFERDISTEIYQAGNKPCNGVAGSNCYSPLQSYGFRPTYGVGHQPYRVVVLSFELLHAPATVCGPKKSTNLVKNKCVNFNFNGLTGTGVLTESNKKFLPFQQFGRDIADTTDAVRDPQTLEILDITPCSFGGVSVITPGTNTSNQVAVLYQGVNCTEVPVAIHADQLTPTWRVYSTGSNVFQTRAGCLIGAEYVNNSYECDIPIGAGICASYQTQTKSHGSASSVASQSIIAYTMSLGAENSVAYSNNSIAIPTNFTISVTTEILPVSMTKTSVDCTMYICGDSTECSNLLLQYGSFCTQLKRALTGIAVEQDKNTQEVFAQVKQIYKTPPIKYFGGFNFSQILPDPSKPSKRSPIEDLLFNKVTLADAGFIKQYGDCLGDIAARDLICAQKFNGLTVLPPLLTDEMIAQYTSALLAGTITSGWTFGAGPALQIPFPMQMAYRFNGIGVTQNVLYENQKLIANQFNSAIGKIQDSLSSTPSALGKLQDVVNHNAQALNTLVKQLSSKFGAISSVLNDILSRLDPPEAEVQIDRLITGRLQSLQTYVTQQLIRAAEIRASANLAATKMSECVLGQSKRVDFCGKGYHLMSFPQSAPHGVVFLHVTYVPAQEKNFTTAPAICHDGKAHFPREGVFVSNGTHWFVTQRNFYEPQIITTDNTFVSGNCDVVIGIVNNTVYDPLQPELDSFKEELDKYFKNHTSPDVDLGDISGINASVVNIQKEIDRLNEVAKNLNESLIDLQELGKYEQYIKWPWYIWLGFIAGLIAIVMVTIMLCCMTSCCSCLKGCCSCGSCCKFDEDDSEPVLKGVKLHYT

SEQ ID NO: 29 - protein, 1269 aa, synthetic construct
MFVFLVLLPLVSSQCVNLITRTQSYTNSFTRGVYYPDKVFRSSVLHSTQDLFLPFFSNVTWFHAIHVSGTNGTKRFDNPALPFNDGVYFASTEKSNIIRGWIFGTTLDSKTQSLLIVNNATNVVIKVCEFQFCNDPFLDVYQKNNKSWMESEFRVYSSANNCTFEYVSQPFLMDLEGKEGNFKNLREFVFKNIDGYFKIYSKHTPINLERDLPQGFSALEPLVDLPIGINITRFQTLLALHRSYLTPVDSSSGWTAGAAAYYVGYLQPRTFLLKYNENGTITDAVDCALDPLSETKCTLKSFTVEKGIYQTSNFRVQPTESIVRFPNITNLCPFHEVFNATTFASVYAWNRKRISNCVADYSVIYNFAPFFAFKCYGVSPTKLNDLCFTNVYADSFVIRGNEVSQIAPGQTGNIADYNYKLPDDFTGCVIAWNSNKLDSKPSGNYNYLYRLFRKSKLKPFERDISTEIYQAGNKPCNGVAGPNCYSPLQSYGFRPTYGVGHQPYRVVVLSFELLHAPATVCGPKKSTNLVKNKCVNFNFNGLTGTGVLTESNKKFLPFQQFGRDIADTTDAVRDPQTLEILDITPCSFGGVSVITPGTNTSNQVAVLYQGVNCTEVPVAIHADQLTPTWRVYSTGSNVFQTRAGCLIGAEYVNNSYECDIPIGAGICASYQTQTKSHRRARSVASQSIIAYTMSLGAENSVAYSNNSIAIPTNFTISVTTEILPVSMTKTSVDCTMYICGDSTECSNLLLQYGSFCTQLKRALTGIAVEQDKNTQEVFAQVKQIYKTPPIKYFGGFNFSQILPDPSKPSKRSFIEDLLFNKVTLADAGFIKQYGDCLGDIAARDLICAQKFNGLTVLPPLLTDEMIAQYTSALLAGTITSGWTFGAGAALQIPFAMQMAYRFNGIGVTQNVLYENQKLIANQFNSAIGKIQDSLSSTASALGKLQDVVNHNAQALNTLVKQLSSKFGAISSVLNDILSRLDKVEAEVQIDRLITGRLQSLQTYVTQQLIRAAEIRASANLAATKMSECVLGQSKRVDFCGKGYHLMSFPQSAPHGVVFLHVTYVPAQEKNFTTAPAICHDGKAHFPREGVFVSNGTHWFVTQRNFYEPQIITTDNTFVSGNCDVVIGIVNNTVYDPLQPELDSFKEELDKYFKNHTSPDVDLGDISGINASVVNIQKEIDRLNEVAKNLNESLIDLQELGKYEQYIKWPWYIWLGFIAGLIAIVMVTIMLCCMTSCCSCLKGCCSCGSCCKFDEDDSEPVLKGVKLHYT

SEQ ID NO: 30 - protein, 1269 aa, synthetic construct
MFVFLVLLPLVSSQCVNLITRTQSYTNSFTRGVYYPDKVFRSSVLHSTQDLFLPFFSNVTWFHAIHVSGTNGTKRFDNPALPFNDGVYFASTEKSNIIRGWIFGTTLDSKTQSLLIVNNATNVVIKVCEFQFCNDPFLDVYQKNNKSWMESEFRVYSSANNCTFEYVSQPFLMDLEGKEGNFKNLREFVFKNIDGYFKIYSKHTPINLERDLPQGFSALEPLVDLPIGINITRFQTLLALHRSYLTPGGSSSGWTAGAAAYYVGYLQPRTFLLKYNENGTITDAVDCALDPLSETKCTLKSFTVEKGIYQTSNFRVQPTESIVRFPNITNLCPFHEVFNATTFASVYAWNRKRISNCVADYSVIYNFAPFFAFKCYGVSPTKLNDLCFTNVYADSFVIRGNEVSQIAPGQTGNIADYNYKLPDDFTGCVIAWNSNKLDSKPSGNYNYLYRLFRKSKLKPFERDISTEIYQAGNKPCNGVAGPNCYSPLQSYGFRPTYGVGHQPYRVVVLSFELLHASATVCGPKKSTNLVKNKCVNFNFNGLTGTGVLTESNKKFLPFQQFGRDIADTTDAVRDPQTLEILDITPCSFGGVSVITPGTNTSNQVAVLYQGVNCTEVPVAIHADQLTPTWRVYSTGSNVFQTRAGCLIGAEYVNNSYECDIPIGAGICASYQTQTKSHGSASSVASQSIIAYTMSLGAENSVAYSNNSIAIPTNFTISVTTEILPVSMTKTSVDCTMYICGDSTECSNLLLQYGSFCTQLKRALTGIAVEQDKNTQEVFAQVKQIYKTPPIKYFGGFNFSQILPDPSKPSKRSPIEDLLFNKVTLADAGFIKQYGDCLGDIAARDLICAQKFNGLTVLPPLLTDEMIAQYTSALLAGTITSGWTFGAGPALQIPFPMQMAYRFNGIGVTQNVLYENQKLIANQFNSAIGKIQDSLSSTPSALGKLQDVVNHNAQALNTLVKQLSSKFGAISSVLNDILSRLDPPEAEVQIDRLITGRLQSLQTYVTQQLIRAAEIRASANLAATKMSECVLGQSKRVDFCGKGYHLMSFPQSAPHGVVFLHVTYVPAQEKNFTTAPAICHDGKAHFPREGVFVSNGTHWFVTQRNFYEPQIITTDNTFVSGNCDVVIGIVNNTVYDPLQPELDSFKEELDKYFKNHTSPDVDLGDISGINASVVNIQKEIDRLNEVAKNLNESLIDLQELGKYEQYIKWPWYIWLGFIAGLIAIVMVTIMLCCMTSCCSCLKGCCSCGSCCKFDEDDSEPVLKGVKLHYT

SEQ ID NO: 31 - DNA, 1479 bp, synthetic construct
  source 1..1479: mol_type = other DNA
atgctactagtaaatcagtcacaccaaggtttcaacaaggaacacaccagcaagatggtgagcgctatcgtgctgtacgtcctgctggccgctgctgctcacagcgctttcgctgctgactccatccacatcaaggacagcgacgacctgaagaaccgtctggccgaggccggtgacaagctggtcgtcatcgacttcatggccacttggtgcggtccttgcaagatgatcggccctaagctggacgagatggctaacgagatgtccgacagcatcgtggtcctgaaggtggacgtcgacgagtgcgaggacatcgccaccgaatacaacatcaacagcatgcccaccttcgtgttcgtgaagaacagcaagaagatcgaggaattttccggcgctaacgtcgacaagctgcgtaacaccatcatcaagctgaagctggccggctccggctccggccacatgcatcaccaccaccaccattcctccggtgacgacgacgacaaggtgcagccaaccgaatctatcgtcagattcccaaacatcactaacctgtgccctttccacgaggtgttcaacgctaccactttcgccagcgtctacgcttggaaccgcaagcgtatcagcaactgcgtcgccgactactctgtgatctacaacttcgctcctttcttcgctttcaagtgctacggcgtgtcacctaccaagctgaacgacctgtgcttcactaacgtctacgccgactccttcgtgatccgcggaaacgaagtctctcagatcgctcctggacagaccggaaatatcgctgactacaactacaagctgccagacgacttcactggctgcgtgatcgcttggaactcaaacaagctggactccaagccttctggcaactacaactacctgtacaggctgttcagaaagtcaaagctgaagcctttcgagcgcgacatctcaaccgaaatctaccaggctggtaatcgaccctgcaacggtgtggctggccctaactgctactctcccctgcagtcctacggtttccgtccaacctacggagtcggtcatcagccttaccgtgtggtcgtgctgagcttcgaactgctccacgctcctgctactgtgtgcggtcccaagaagtctactaacctggtcaaaaacaaaagcgtcaacttcaacttcaacggtctgtacgagaaccagaagctgatcgctaaccagttcaacagcgccatcggcaagatccaggactcactgtcatccactgcctccgctctgggaaagctgcaggacgtcgtgaaccagaacgcccaggctctgaacaccctggtcaagcagctgaagaaccacacctctcctgacgtcgacctgggcgacatcagcggaatcaacgcttctgtcgtgaacatccagaaggagatcgaccgcctgaacgaagtggccaagaacctgaacgaatccctgattgacctccaagaactctaa

SEQ ID NO: 32 - DNA, 1479 bp, synthetic construct
  source 1..1479: mol_type = other DNA
atgctactagtaaatcagtcacaccaaggtttcaacaaggaacacaccagcaagatggtgagcgctatcgtgctgtacgtcctgctggccgctgctgctcacagcgctttcgctgctgactccatccacatcaaggacagcgacgacctgaagaaccgtctggccgaggccggtgacaagctggtcgtcatcgacttcatggccacttggtgcggtccttgcaagatgatcggccctaagctggacgagatggctaacgagatgtccgacagcatcgtggtcctgaaggtggacgtcgacgagtgcgaggacatcgccaccgaatacaacatcaacagcatgcccaccttcgtgttcgtgaagaacagcaagaagatcgaggaattttccggcgctaacgtcgacaagctgcgtaacaccatcatcaagctgaagctggccggctccggctccggccacatgcatcaccaccaccaccattcctccggtgacgacgacgacaaggtgcagccaaccgaatctatcgtcagattcccaaacatcactaacctgtgccctttccacgaggtgttcaacgctaccactttcgccagcgtctacgcttggaaccgcaagcgtatcagcaactgcgtcgccgactactctgtgatctacaacttcgctcctttcttcgctttcaagtgctacggcgtgtcacctaccaagctgaacgacctgtgcttcactaacgtctacgccgactccttcgtgatccgcggaaacgaagtctctcagatcgctcctggacagaccggaaatatcgctgactacaactacaagctgccagacgacttcactggctgcgtgatcgcttggaactcaaacaagctggactccaagccttctggcaactacaactacctgtacaggctgttcagaaagtcaaagctgaagcctttcgagcgcgacatctcaaccgaaatctaccaggctggtaataagccctgcaacggtgtggctggctctaactgctactctcccctgcagtcctacggtttccgtccaacctacggagtcggtcatcagccttaccgtgtggtcgtgctgagcttcgaactgctccacgctcctgctactgtgtgcggtcccaagaagtctactaacctggtcaaaaacaaaagcgtcaacttcaacttcaacggtctgtacgagaaccagaagctgatcgctaaccagttcaacagcgccatcggcaagatccaggactcactgtcatccactgcctccgctctgggaaagctgcaggacgtcgtgaaccagaacgcccaggctctgaacaccctggtcaagcagctgaagaaccacacctctcctgacgtcgacctgggcgacatcagcggaatcaacgcttctgtcgtgaacatccagaaggagatcgaccgcctgaacgaagtggccaagaacctgaacgaatccctgattgacctccaagaactctaa

SEQ ID NO: 33 - DNA, 1185 bp, synthetic construct
  source 1..1185: mol_type = other DNA
atgctactagtaaatcagtcacaccaaggtttcaacaaggaacacaccagcaagatggtgagcgctatcgtgctgtacgtcctgctggccgctgctgctcacagcgctttcgctgctgactccatccacatcaaggacagcgacgacctgaagaaccgtctggccgaggccggtgacaagctggtcgtcatcgacttcatggccacttggtgcggtccttgcaagatgatcggccctaagctggacgagatggctaacgagatgtccgactgcatcgtggtcctgaaggtggacgtcgacgagtgcgaggacatcgccaccgaatacaacatcaacagcatgcccaccttcgtgttcgtgaagaacagcaagaagatcgaggaattttccggcgctaacgtcgacaagctgcgtaacaccatcatcaagctgaagctggccggctccggctccggccacatgcatcaccaccaccaccattcctccggtgacgacgacgacaaggtgcagccaaccgaatctatcgtcagattcccaaacatcactaacctgtgccctttccacgaggtgttcaacgctaccactttcgccagcgtctacgcttggaaccgcaagcgtatcagcaactgcgtcgccgactactctgtgatctacaacttcgctcctttcttcgctttcaagtgctacggcgtgtcacctaccaagctgaacgacctgtgcttcactaacgtctacgccgactccttcgtgatccgcggaaacgaagtctctcagatcgctcctggacagaccggaaatatcgctgactacaactacaagctgccagacgacttcactggctgcgtgatcgcttggaactcaaacaagctggactccaagccttctggcaactacaactacctgtacaggctgttcagaaagtcaaagctgaagcctttcgagcgcgacatctcaaccgaaatctaccaggctggtaataagccctgcaacggtgtggctggccctaactgctactctcccctgcagtcctacggtttccgtccaacctacggagtcggtcatcagccttaccgtgtggtcgtgctgagcttcgaactgctccacgctcctgctactgtgtgcggtcccaagaagtctactaacctggtcaaaaacaaatgtgtcaacttcaacttcaacggttaa

SEQ ID NO: 34 - DNA, 1185 bp, synthetic construct
  source 1..1185: mol_type = other DNA
atgctactagtaaatcagtcacaccaaggtttcaacaaggaacacaccagcaagatggtgagcgctatcgtgctgtacgtcctgctggccgctgctgctcacagcgctttcgctgctgactccatccacatcaaggacagcgacgacctgaagaaccgtctggccgaggccggtgacaagctggtcgtcatcgacttcatggccacttggtgcggtccttgcaagatgatcggccctaagctggacgagatggctaacgagatgtccgactgcatcgtggtcctgaaggtggacgtcgacgagtgcgaggacatcgccaccgaatacaacatcaacagcatgcccaccttcgtgttcgtgaagaacagcaagaagatcgaggaattttccggcgctaacgtcgacaagctgcgtaacaccatcatcaagctgaagctggccggctccggctccggccacatgcatcaccaccaccaccattcctccggtgacgacgacgacaaggtgcagccaaccgaatctatcgtcagattcccaaacatcactaacctgtgccctttccacgaggtgttcaacgctaccactttcgccagcgtctacgcttggaaccgcaagcgtatcagcaactgcgtcgccgactactctgtgatctacaactccgctagcttctctgctttcaagtgctacggcgtgtcacctaccaagctgaacgacctgtgcttcactaacgtctacgccgactccttcgtgatccgcggaaacgaagtctctcagatcgctcctggacagaccggaaatatcgctgactacaactacaagctgccagacgacttcactggctgcgtgatcgcttggaactcaaacaagctggactccaagccttctggcaactacaactacctgtacaggctgttcagaaagtcaaagctgaagcctttcgagcgcgacatctcaaccgaaatctaccaggctggtaataagccctgcaacggtgtggctggccctaactgctactctcccctgcagtcctacggtttccgtccaacctacggagtcggtcatcagccttaccgtgtggtcgtgctgagcttcgaactgctccacgctcctgctactgtgtgcggtcccaagaagtctactaacctggtcaaaaacaaatgtgtcaacttcaacttcaacggttaa

SEQ ID NO: 35 - DNA, 1479 bp, synthetic construct
  source 1..1479: mol_type = other DNA
atgctgctggtgaaccagagccaccagggtttcaacaaggaacacactagcaagatggtgtctgctatcgtcctctacgtgctgctcgccgccgctgctcactcagctttcgccgctgactctatccacatcaaggactccgacgacctcaagaaccgtttggccgaagccggcgacaagctggtcgttatcgacttcatggctacctggtgtggcccttgcaagatgatcggacctaagctggacgaaatggctaacgagatgagcgacagcatcgtcgttctgaaggtggacgtcgacgaatgtgaggacatcgccactgagtacaacatcaacagcatgcctaccttcgttttcgtgaagaactctaagaagatcgaggagttctctggtgccaacgtggacaagctccgtaacaccatcatcaagctcaagctggccggcagcggtagcggtcacatgcaccaccaccaccaccattcaagcggcgacgacgacgacaaggtgcagccaaccgaatcaatcgtccgcttcccaaacatcactaacctgtgcccattccacgaggtgttcaacgccaccactttcgcctctgtctacgcttggaaccgcaagcgcatctccaactgtgtcgccgactacagcgtgatatacaacttcgctcctttcttcgcattcaagtgttacggagtgtcccctaccaagctcaacgatttgtgcttcacaaacgtgtacgctgacagcttcgtgatccgtggtaacgaggtttctcaaatcgcccctggtcagacaggtaacatcgctgactacaactacaagctcccagacgacttcactggctgtgttatcgcttggaactcaaacaagctggactctaagccgtctggtaactacaactacctctaccgtctgttccgcaagagcaagctcaagccattcgaacgtgacatcagcacagagatctaccaagccggtaacaagccctgcaacggcgttgccggacctaactgctactctcccctccagtcctacggattccgcccaacctacggcgtgggtcaccagccataccgcgtggttgtgctgagcttcgaactgctgcacgcccccgctaccgtgtgtggccctaagaagagcactaacctcgttaagaacaagtccgtgaacttcaacttcaacggtctctacgaaaaccagaagctgatcgctaaccagttcaactccgccatcggcaagatccaggactccctgtcctccacagcttccgctctgggcaagctgcaggacgttgtgaaccaaaacgctcaggccctgaacacactggtgaagcaactgaagaaccacaccagccccgacgttgacctgggtgacatcagcggtatcaacgctagcgtggtgaacatccagaaggagatcgacaggctgaacgaagtggctaagaacttgaacgagagcctcatcgacctgcaggaactgtaa

SEQ ID NO: 36 - DNA, 1479 bp, synthetic construct
  source 1..1479: mol_type = other DNA
atgctgctggtgaaccagagccaccagggtttcaacaaggaacacactagcaagatggtgtctgctatcgtcctctacgtgctgctcgccgccgctgctcactcagctttcgccgctgactctatccacatcaaggactccgacgacctcaagaaccgtttggccgaagccggcgacaagctggtcgttatcgacttcatggctacctggtgtggcccttgcaagatgatcggacctaagctggacgaaatggctaacgagatgagcgacagcatcgtcgttctgaaggtggacgtcgacgaatgtgaggacatcgccactgagtacaacatcaacagcatgcctaccttcgttttcgtgaagaactctaagaagatcgaggagttctctggtgccaacgtggacaagctccgtaacaccatcatcaagctcaagctggccggcagcggtagcggtcacatgcaccaccaccaccaccattcaagcggcgacgacgacgacaaggtgcagccaaccgaatcaatcgtccgcttcccaaacatcactaacctgtgcccattccacgaggtgttcaacgccaccactttcgcctctgtctacgcttggaaccgcaagcgcatctccaactgtgtcgccgactacagcgtgatatacaactccgcttctttctctgcattcaagtgttacggagtgtcccctaccaagctcaacgatttgtgcttcacaaacgtgtacgctgacagcttcgtgatccgtggtaacgaggtttctcaaatcgcccctggtcagacaggtaacatcgctgactacaactacaagctcccagacgacttcactggctgtgttatcgcttggaactcaaacaagctggactctaagccgtctggtaactacaactacctctaccgtctgttccgcaagagcaagctcaagccattcgaacgtgacatcagcacagagatctaccaagccggtaacaagccctgcaacggcgttgccggacctaactgctactctcccctccagtcctacggattccgcccaacctacggcgtgggtcaccagccataccgcgtggttgtgctgagcttcgaactgctgcacgcccccgctaccgtgtgtggccctaagaagagcactaacctcgttaagaacaagtccgtgaacttcaacttcaacggtctctacgaaaaccagaagctgatcgctaaccagttcaactccgccatcggcaagatccaggactccctgtcctccacagcttccgctctgggcaagctgcaggacgttgtgaaccaaaacgctcaggccctgaacacactggtgaagcaactgaagaaccacaccagccccgacgttgacctgggtgacatcagcggtatcaacgctagcgtggtgaacatccagaaggagatcgacaggctgaacgaagtggctaagaacttgaacgagagcctcatcgacctgcaggaactgtaa

SEQ ID NO: 37 - DNA, 1185 bp, synthetic construct
  source 1..1185: mol_type = other DNA
atgctactagtaaatcagtcacaccaaggtttcaacaaggaacacaccagcaagatggtgagcgctatcgtgctgtacgtcctgctggccgctgctgctcacagcgctttcgctgctgactccatccacatcaaggacagcgacgacctgaagaaccgtctggccgaggccggtgacaagctggtcgtcatcgacttcatggccacttggtgcggtccttgcaagatgatcggccctaagctggacgagatggctaacgagatgtccgactgcatcgtggtcctgaaggtggacgtcgacgagtgcgaggacatcgccaccgaatacaacatcaacagcatgcccaccttcgtgttcgtgaagaacagcaagaagatcgaggaattttccggcgctaacgtcgacaagctgcgtaacaccatcatcaagctgaagctggccggctccggctccggccacatgcatcaccaccaccaccattcctccggtgacgacgacgacaaggtgcagccaaccgaatctatcgtcagattcccaaacatcactaacctgtgccctttccacgaggtgttcaacgctaccactttcgccagcgtctacgcttggaaccgcaagcgtatcagcaactgcgtcgccgactactctgtgatctacaacttcgctcctttcttcgctttcaagtgctacggcgtgtcacctaccaagctgaacgacctgtgcttcactaacgtctacgccgactccttcgtgatccgcggaaacgaagtctctcagatcgctcctggacagaccggaaatatcgctgactacaactacaagctgccagacgacttcactggctgcgtgatcgcttggaactcaaacaagctggactccaagccttctggcaactacaactacctgtacaggctgttcagaaagtcaaagctgaagcctttcgagcgcgacatctcaaccgaaatctaccaggctggtaataagccctgcaacggtgtggctggccctaactgctactctcccctgcagtcctacggtttccgtccaacctacggagtcggtcatcagccttaccgtgtggtcgtgctgagcttcgaactgctccacgcttctgctactgtgtgcggtcccaagaagtctactaacctggtcaaaaacaaatgtgtcaacttcaacttcaacggttaa

SEQ ID NO: 38 - DNA, 1479 bp, synthetic construct
  source 1..1479: mol_type = other DNA
atgctgctggtgaaccagagccaccagggtttcaacaaggaacacactagcaagatggtgtctgctatcgtcctctacgtgctgctcgccgccgctgctcactcagctttcgccgctgactctatccacatcaaggactccgacgacctcaagaaccgtttggccgaagccggcgacaagctggtcgttatcgacttcatggctacctggtgtggcccttgcaagatgatcggacctaagctggacgaaatggctaacgagatgagcgacagcatcgtcgttctgaaggtggacgtcgacgaatgtgaggacatcgccactgagtacaacatcaacagcatgcctaccttcgttttcgtgaagaactctaagaagatcgaggagttctctggtgccaacgtggacaagctccgtaacaccatcatcaagctcaagctggccggcagcggtagcggtcacatgcaccaccaccaccaccattcaagcggcgacgacgacgacaaggtgcagccaaccgaatcaatcgtccgcttcccaaacatcactaacctgtgcccattccacgaggtgttcaacgccaccactttcgcctctgtctacgcttggaaccgcaagcgcatctccaactgtgtcgccgactacagcgtgatatacaacttcgctcctttcttcgcattcaagtgttacggagtgtcccctaccaagctcaacgatttgtgcttcacaaacgtgtacgctgacagcttcgtgatccgtggtaacgaggtttctcaaatcgcccctggtcagacaggtaacatcgctgactacaactacaagctcccagacgacttcactggctgtgttatcgcttggaactcaaacaagctggactctaagccgtctggtaactacaactacctctaccgtctgttccgcaagagcaagctcaagccattcgaacgtgacatcagcacagagatctaccaagccggtaacaagccctgcaacggcgttgccggacctaactgctactctcccctccagtcctacggattccgcccaacctacggcgtgggtcaccagccataccgcgtggttgtgctgagcttcgaactgctgcacgcctccgctaccgtgtgtggccctaagaagagcactaacctcgttaagaacaagtccgtgaacttcaacttcaacggtctctacgaaaaccagaagctgatcgctaaccagttcaactccgccatcggcaagatccaggactccctgtcctccacagcttccgctctgggcaagctgcaggacgttgtgaaccaaaacgctcaggccctgaacacactggtgaagcaactgaagaaccacaccagccccgacgttgacctgggtgacatcagcggtatcaacgctagcgtggtgaacatccagaaggagatcgacaggctgaacgaagtggctaagaacttgaacgagagcctcatcgacctgcaggaactgtaa

SEQ ID NO: 39 - DNA, 1479 bp, synthetic construct
  source 1..1479: mol_type = other DNA
atgctgctggtgaaccagagccaccagggtttcaacaaggaacacactagcaagatggtgtctgctatcgtcctctacgtgctgctcgccgccgctgctcactcagctttcgccgctgactctatccacatcaaggactccgacgacctcaagaaccgtttggccgaagccggcgacaagctggtcgttatcgacttcatggctacctggtgtggcccttgcaagatgatcggacctaagctggacgaaatggctaacgagatgagcgacagcatcgtcgttctgaaggtggacgtcgacgaatgtgaggacatcgccactgagtacaacatcaacagcatgcctaccttcgttttcgtgaagaactctaagaagatcgaggagttctctggtgccaacgtggacaagctccgtaacaccatcatcaagctcaagctggccggcagcggtagcggtcacatgcaccaccaccaccaccattcaagcggcgacgacgacgacaaggtgcagccaaccgaatcaatcgtccgcttcccaaacatcactaacctgtgcccattccacgaggtgttcaacgccaccactttcgcctctgtctacgcttggaaccgcaagcgcatctccaactgtgtcgccgactacagcgtgatatacaacttcgctcctttcttcgcattcaagtgttacggagtgtcccctaccaagctcaacgatttgtgcttcacaaacgtgtacgctgacagcttcgtgatccgtggtaacgaggtttctcaaatcgcccctggtcagacaggtaacatcgctgactacaactacaagctcccagacgacttcactggctgtgttatcgcttggaactcaaacaagctggactctaagccgtctggtaactacaactacctctaccgtctgctccgcaagagcaagctcaagccattcgaacgtgacatcagcacagagatctaccaagccggtaaccgcccctgcaacggcgttgccggacctaactgctactctcccctccagtcctacggattccgcccaacctacggcgtgggtcaccagccataccgcgtggttgtgctgagcttcgaactgctgcacgcccccgctaccgtgtgtggccctaagaagagcactaacctcgttaagaacaagtccgtgaacttcaacttcaacggtctctacgaaaaccagaagctgatcgctaaccagttcaactccgccatcggcaagatccaggactccctgtcctccacagcttccgctctgggcaagctgcaggacgttgtgaaccaaaacgctcaggccctgaacacactggtgaagcaactgaagaaccacaccagccccgacgttgacctgggtgacatcagcggtatcaacgctagcgtggtgaacatccagaaggagatcgacaggctgaacgaagtggctaagaacttgaacgagagcctcatcgacctgcaggaactgtaa

SEQ ID NO: 40 - DNA, 1476 bp, synthetic construct
  source 1..1476: mol_type = other DNA
atgctgctggtgaaccagagccaccagggtttcaacaaggaacacactagcaagatggtgtctgctatcgtcctctacgtgctgctcgccgccgctgctcactcagctttcgccgctgactctatccacatcaaggactccgacgacctcaagaaccgtttggccgaagccggcgacaagctggtcgttatcgacttcatggctacctggtgtggcccttgcaagatgatcggacctaagctggacgaaatggctaacgagatgagcgacagcatcgtcgttctgaaggtggacgtcgacgaatgtgaggacatcgccactgagtacaacatcaacagcatgcctaccttcgttttcgtgaagaactctaagaagatcgaggagttctctggtgccaacgtggacaagctccgtaacaccatcatcaagctcaagctggccggcagcggtagcggtcacatgcaccaccaccaccaccattcaagcggcgacgacgacgacaaggtgcagccaaccgaatcaatcgtccgcttcccaaacgtcactaacctgtgcccattccacgaggtgttcaacgccacccgtttcgcctctgtctacgcttggaaccgcacgcgcatctccaactgtgtcgccgactacagcgtgctgtacaacttcgctcctttcttcgcattcaagtgttacggagtgtcccctaccaagctcaacgatttgtgcttcacaaacgtgtacgctgacagcttcgtgatcaagggtaacgaggtttctcaaatcgcccctggtcagacaggtaacatcgctgactacaactacaagctcccagacgacttcactggctgtgttatcgcttggaactcaaacaagctggactctaagcattctggtaactacgactactggtaccgtctgttccgcaagagcaagctcaagccattcgaacgtgacatcagcacagagatctaccaagccggtaacaagccctgcaagggcaagggacctaactgctacttccccctccagtcctacggattccgcccaacctacggcgtgggtcaccagccataccgcgtggttgtgctgagcttcgaactgctgcacgcccccgctaccgtgtgtggccctaagaagagcactaacctcgttaagaacaagtccgtgaacttcaacttcaacggtctctacgaaaaccagaagctgatcgctaaccagttcaactccgccatcggcaagatccaggactccctgtcctccacagcttccgctctgggcaagctgcaggacgttgtgaaccaaaacgctcaggccctgaacacactggtgaagcaactgaagaaccacaccagccccgacgttgacctgggtgacatcagcggtatcaacgctagcgtggtgaacatccagaaggagatcgacaggctgaacgaagtggctaagaacttgaacgagagcctcatcgacctgcaggaactgtaa

SEQ ID NO: 41 - DNA, 1479 bp, synthetic construct
  source 1..1479: mol_type = other DNA
atgctgctggtgaaccagagccaccagggtttcaacaaggaacacactagcaagatggtgtctgctatcgtcctctacgtgctgctcgccgccgctgctcactcagctttcgccgctgactctatccacatcaaggactccgacgacctcaagaaccgtttggccgaagccggcgacaagctggtcgttatcgacttcatggctacctggtgtggcccttgcaagatgatcggacctaagctggacgaaatggctaacgagatgagcgacagcatcgtcgttctgaaggtggacgtcgacgaatgtgaggacatcgccactgagtacaacatcaacagcatgcctaccttcgttttcgtgaagaactctaagaagatcgaggagttctctggtgccaacgtggacaagctccgtaacaccatcatcaagctcaagctggccggcagcggtagcggtcacatgcaccaccaccaccaccattcaagcggcgacgacgacgacaaggtgcagccaaccgaatcaatcgtccgcttcccaaacatcactaacctgtgcccattccacgaggtgttcaacgccaccactttcgcctctgtctacgcttggaaccgcaagcgcatctccaactgtgtcgccgactacagcgtgatatacaacttcgctcctttcttcgcattcaagtgttacggagtgtcccctaccaagctcaacgatttgtgcttcacaaacgtgtacgctgacagcttcgtgatccgtggtaacgaggtttctcaaatcgcccctggtcagacaggtaacatcgctgactacaactacaagctcccagacgacttcactggctgtgttatcgcttggaactcaaacaagctggactctaagccgtctggtaactacaactacctctaccgtctgctccgcaagagcaagctcaagccattcgaacgtgacatcagcacagagatctaccaagccggtaacaagccctgcaacggcgttgccggacctaactgctactctcccctccagtcctacggattccgcccaacctacggcgtgggtcaccagccataccgcgtggttgtgctgagcttcgaactgctgcacgcccccgctaccgtgtgtggccctaagaagagcactaacctcgttaagaacaagtccgtgaacttcaacttcaacggtctctacgaaaaccagaagctgatcgctaaccagttcaactccgccatcggcaagatccaggactccctgtcctccacagcttccgctctgggcaagctgcaggacgttgtgaaccaaaacgctcaggccctgaacacactggtgaagcaactgaagaaccacaccagccccgacgttgacctgggtgacatcagcggtatcaacgctagcgtggtgaacatccagaaggagatcgacaggctgaacgaagtggctaagaacttgaacgagagcctcatcgacctgcaggaactgtaa

SEQ ID NO: 42 - DNA, 3810 bp, synthetic construct
  source 1..3810: mol_type = other DNA
atgttcgtgttcctggtgctgctgcccctggtgagcagccaatgcgtgaacctgatcacaagaacacagagctacaccaacagcttcacaagaggcgtgtactaccccgacaaggtgttcagaagcagcgtgctgcattccacccaagacctgttcctgcccttcttcagcaacgtgacctggttccacgccatccacgtgagcggcaccaacggcaccaagagattcgacaaccccgccctgcccttcaacgacggcgtgtacttcgctagcaccgagaagagcaacatcatcagaggctggatcttcggcaccaccctggacagcaaaacacagagcctgctgatcgtgaacaatgccaccaacgtggtgatcaaggtgtgcgagtttcagttctgcaacgaccccttcctggacgtgtatcagaagaacaacaagagctggatggagagcgagttcagagtgtacagcagcgccaacaactgcaccttcgagtacgtgagccaacccttcctgatggacctggtgggcaaggagggcaactttaagaacctcagagagttcgtgttcaagaacatcgacggctacttcaagatctacagcaagcacacccccatcaacctggagagagacctgccccaaggcttcagcgccctggagcccctggtggacctgcccatcggcatcaacatcacaagatttcagaccctgctggccctgcacagaagctatctcacacccgtcgatagcagcagcgggtggacagccggggccgctgcctactacgtgggctacctgcagcctagaaccttcctgctgaagtacaacgagaacggcacaatcaccgacgccgtcgactgcgccctggaccccctgagcgagaccaagtgcaccctgaagagcttcaccgtggagaagggcatctatcagacaagcaacttcagagtgcagcccaccgagagcatcgtgagattccccaacatcaccaacctgtgccccttccacgaggtgttcaacgccaccaccttcgctagcgtgtacgcttggaatagaaagagaatcagcaactgcgtggccgactacagcgtgatctacaacttcgcccccttcttcgccttcaagtgttacggcgtgtcccccaccaagctgaacgacctgtgcttcaccaacgtgtacgccgacagcttcgtgatcagaggcaacgaggtgagccaaatcgcccctgggcagaccggcaacatcgccgactacaactacaagctgcccgacgacttcaccggctgcgtgatcgcctggaacagcaacaagctggactccaagcctagcgggaattacaactacctgtacagactgttcagaaagagcaagctgaagcccttcgagagagacatcagcaccgagatctaccaagccggcaacagaccctgcaacggcgtggccggccccaactgctacagccccctgcagagctacggcttcagacccacctacggcgtgggccatcagccctacagagtggtcgtgctgagcttcgagctgctgcacgcccccgccaccgtgtgcggccccaagaagagcaccaacctggtgaagaacaagtgcgtgaacttcaacttcaacgggctgaccggcaccggcgtgctgaccgagagcaacaagaagttcctgccctttcaacagttcggcagagacatcgccgacaccaccgatgccgtgagagaccctcagaccctggagatcctggacatcaccccctgcagcttcggcggcgtgagcgtgatcacccccggcaccaacacaagcaaccaagtggccgtgctgtaccaaggcgtgaactgcaccgaggtgcccgtggccatccacgccgatcagctgacccccacctggagagtgtatagcaccggcagcaacgtgtttcagacaagagccggctgcctgatcggcgccgagtacgtgaacaacagctacgagtgcgacatccccatcggcgccggcatctgcgctagctatcagacacagaccaagagccacggcagcgctagcagcgtggctagccaaagcatcatcgcctacaccatgagcctgggcgccgagaacagcgtggcctacagcaacaacagcatcgccatccccaccaacttcaccatcagcgtgaccaccgaaattctgcccgtgagcatgaccaagacaagcgtggactgcaccatgtacatctgcggcgacagcaccgagtgcagcaacctgctcctgcagtacggcagcttctgcacacagctgaagagagccctgaccggcatcgccgtggagcaagacaagaacacccaagaggtgttcgcccaagtgaagcagatctacaagaccccccccatcaagtacttcggcggcttcaacttcagccaaatcctgcccgaccctagcaagccctccaagagaagccccatcgaggacctgctgttcaacaaggtgaccctggccgacgccggcttcatcaagcagtacggcgactgcctcggcgacatcgctgctagagacctgatctgcgctcagaagttcaacgggctcaccgtgctgccccccctgctgaccgacgagatgattgctcagtacacctccgccctgctggccggcaccatcacaagcggctggacctttggggctggccccgccctgcagatccccttccccatgcagatggcctacagattcaacggcatcggcgtgacacagaacgtgctgtacgagaatcagaagctgatcgccaatcagttcaacagcgccatcggcaagatccaagacagcctgagcagcacccctagcgccctgggcaagctgcaagacgtggtgaaccacaacgcccaagccctgaacaccctggtgaagcagctgagcagcaagttcggcgccatcagcagcgtgctgaacgatatcctgagcagactggacccccccgaggccgaggtgcagatcgatagactgatcaccggcagactgcagagcctgcagacctacgtgacacagcagctgatcagagccgccgagatcagagctagcgccaacctggccgccaccaagatgagcgagtgcgtgctggggcagagcaagagagtggacttctgcggcaagggctaccacctgatgagcttccctcagagcgccccccacggcgtggtgttcctgcacgtgacctacgtgcccgcccaagagaagaacttcacaaccgcccccgccatctgccacgacggcaaggcccacttccctagagagggcgtgttcgtgagcaacggcacccactggttcgtgacacagagaaacttctacgagcctcagatcatcaccaccgacaacaccttcgtgagcggcaactgcgacgtggtgatcgggattgtcaacaacaccgtgtacgaccccctgcaacctgagctggacagcttcaaggaggagctggacaagtacttcaagaaccacacaagccccgacgtggacctgggcgacatttccggcatcaacgctagcgtggtgaacattcagaaggagatcgacagactgaatgaggtggccaagaacctgaacgagagcctgatcgacctgcaagagctgggcaagtacgagcagtacatcaagtggccctggtacatctggctgggcttcatcgccggcctgatcgccatcgtgatggtgaccatcatgctgtgctgcatgacaagctgctgtagctgcctgaagggctgctgcagctgcggctcctgctgcaagttcgacgaggacgacagcgagcccgtgctgaagggcgtgaagctgcactacacctga

SEQ ID NO: 43 - DNA, 3810 bp, synthetic construct
  source 1..3810: mol_type = other DNA
atgttcgtgttcctggtgctgctgcccctggtgagcagccaatgcgtgaacctgatcacaagaacacagagctacaccaacagcttcacaagaggcgtgtactaccccgacaaggtgttcagaagcagcgtgctgcattccacccaagacctgttcctgccctttttcagcaacgtgacctggttcagagccatccacgtgagcggcaccaacggcaccaagagattcgacaaccccgccctgcccttcaacgacggcgtgtacttcgctagcaccgagaagagcaacatcatcagaggctggatcttcggcaccaccctggacagcaagacacagagcctgctgatcgtgaacaacgccaccaacgtggtgatcaaggtgtgcgagtttcagttctgcaacgaccccttcctggacgtgtatcagaagaacaacaagagctggatggagagcgagttcagagtgtacagcagcgccaacaactgcaccttcgagtacgtgagccaacccttcctgatggacctggagggcaaggagggcaacttcaagaacctcagagagttcgtgttcaagaacatcgacggctacttcaagatctacagcaagcacacccccatcaacctggagagagacctgccccaaggcttcagcgccctggagcccctggtggacctgcccatcggcatcaacatcacaagatttcagaccctgctggctctgcaccggagctacctgacccctggcggcagcagcagcgggtggaccgccggcgccgctgcctactacgtgggctacctgcagcctagaaccttcctgctgaagtacaacgagaacggcaccattaccgatgccgtggactgtgccctggaccccctgagcgagaccaagtgcaccctgaagagcttcaccgtggagaagggcatctatcagacaagcaacttcagagtgcagcccaccgagagcatcgtgagattccccaacatcaccaacctgtgccccttccacgaggtgttcaacgccaccaccttcgctagcgtgtacgcctggaaccggaagagaatcagcaactgcgtggccgactacagcgtgatctacaacttcgcccccttcttcgccttcaagtgttacggggtgagccccaccaagctgaacgacctgtgcttcaccaacgtgtacgccgacagcttcgtgatcagaggcaacgaggtgagccaaatcgcccctgggcagaccggcaacatcgccgactacaactacaagctgcccgacgacttcaccggctgcgtgatcgcctggaactccaacaagctcgacagcaagcctagcggcaactacaactacctgtacagactgttcagaaagagcaagctgaagcccttcgagagagacatcagcaccgagatctaccaagccggcaacaagccctgcaacggcgtggccggcagcaactgctacagccccctgcagagctacggcttcagacccacctacggcgtgggccatcagccctacagagtggtcgtgctgagcttcgagctgctgcacgcccccgccaccgtgtgcggccccaagaagagcaccaacctggtgaagaacaagtgcgtgaacttcaactttaacggcctgaccggcaccggcgtgctgaccgagagcaacaagaagttcctgcctttccaacagttcggcagagacatcgccgacaccaccgacgccgtgagagaccctcagaccctggagatcctggacatcaccccttgcagcttcggcggcgtgagcgtgatcacccccggcaccaacacaagcaaccaagtggccgtgctgtaccaaggcgtgaactgcaccgaggtgcccgtggccatccacgccgatcagctgacccccacctggcgggtgtacagcaccgggagcaacgtgtttcagacaagagccggctgcctgatcggcgccgagtacgtgaacaacagctacgagtgcgacatccccatcggcgccggcatctgcgctagctatcagacacagaccaagagccacggcagcgctagcagcgtggctagccaaagcatcatcgcctacaccatgagcctgggcgccgagaacagcgtggcctacagcaacaacagcatcgccatccccaccaacttcaccatcagcgtgaccaccgagatcctgcccgtgagcatgaccaagacaagcgtggactgcaccatgtacatctgcggcgacagcaccgagtgcagcaacctgctcctgcagtacggcagcttctgcacacagctgaagagagccctgaccggcatcgccgtggagcaagacaagaacacccaagaggtgttcgcccaagtgaagcagatctacaagaccccccccatcaagtacttcggcggcttcaacttcagccaaatcctccccgaccctagcaagccctccaagagaagccccatcgaggacctgctgttcaacaaggtgaccctggccgacgccggcttcatcaagcagtacggcgactgcctgggcgatatcgccgctagagacctgatctgcgctcagaagttcaacggcctgaccgtcctgccccccctgctgaccgacgagatgatcgcccaatatacatccgccctcctggccggcaccatcacatccgggtggacctttggggccgggcctgccctgcagatccccttccccatgcagatggcctacagattcaacggcatcggcgtgacacagaacgtgctgtacgagaatcagaagctgatcgccaatcagttcaacagcgccatcggcaagatccaagacagcctgagcagcacccctagcgccctgggcaagctgcaagacgtggtgaaccacaacgcccaagccctgaacaccctggtgaagcagctgagcagcaagttcggcgccatcagctccgtgctgaacgacatcctgagcagactggacccccccgaggccgaggtgcaaatcgacagactgatcaccggcagactgcagagcctgcagacctacgtgacacagcagctgatcagagccgccgagatcagagctagcgccaacctggccgccaccaagatgagcgagtgcgtgctggggcagagcaagagagtggacttctgcggcaagggctaccacctgatgagcttccctcagagcgccccccacggcgtggtgttcctgcacgtgacctacgtgcccgcccaagagaagaacttcaccacagcccccgccatctgccacgacggcaaggcccacttccctagagagggcgtgttcgtgagcaacggcacccactggttcgtgacacagagaaacttctacgagcctcagatcatcaccaccgacaacaccttcgtgagcggcaactgcgacgtggtgatcggcatcgtgaacaatacagtgtacgaccccctgcagcccgagctggacagcttcaaggaggagctggacaagtacttcaaaaaccacacaagccccgacgtggacctgggcgacatctccggcatcaacgctagcgtggtgaacattcagaaggagatcgatagactgaacgaggtggccaagaacctgaacgagagcctgatcgacctgcaagagctgggcaagtacgagcagtacatcaagtggccctggtacatctggctgggcttcatcgccggcctgatcgccatcgtgatggtgaccatcatgctgtgctgcatgacaagctgctgcagctgcctgaaaggctgctgtagctgcggcagctgctgcaagttcgacgaggacgacagcgagcccgtgctgaagggcgtgaagctgcactacacctga

SEQ ID NO: 44 - DNA, 3810 bp, synthetic construct
  source 1..3810: mol_type = other DNA
atgttcgtgttcctggtgctgctgcccctggtgagcagccaatgcgtgaacctgatcacaagaacacagagctacaccaacagcttcacaagaggcgtgtactaccccgacaaggtgttcagaagcagcgtgctgcattccacccaagacctgttcctccccttcttttccaacgtgacctggttccacgccatccacgtgagcggcaccaacggcaccaagagattcgacaaccccgccctgcccttcaacgacggcgtgtacttcgctagcaccgagaagagcaacatcatcagaggctggatcttcggcaccaccctggacagcaagacacagagcctgctgatcgtgaacaatgccaccaacgtggtgatcaaggtgtgcgagtttcagttctgcaacgaccccttcctggacgtgtatcagaagaacaacaagagctggatggagagcgagttcagagtgtacagcagcgctaacaactgcaccttcgagtacgtgagccaacccttcctgatggacctggagggcaaggagggcaacttcaagaacctcagagagttcgtgttcaagaacatcgacggctacttcaagatctacagcaagcacacccccatcaacctggagagagacctgccccaaggcttcagcgccctggagcccctggtggacctgcccatcggcatcaacatcacaagatttcagaccctgctggccctgcacagaagctatctgacacctgtggacagcagcagcggctggacagctggggccgctgcctactacgtgggctacctgcagcctagaaccttcctgctgaagtacaacgagaacggcacaatcaccgatgccgtggattgcgccctggaccccctgagcgagaccaagtgcaccctgaagagcttcaccgtggagaagggcatctatcagacaagcaacttcagagtgcagcccaccgagagcatcgtgagattccccaacatcaccaacctgtgccccttccacgaggtgttcaacgccaccaccttcgctagcgtgtacgcttggaacagaaaaagaatcagcaactgcgtggccgactacagcgtgatctacaacttcgcccccttcttcgccttcaagtgctacggggtgagccccaccaagctgaacgacctgtgcttcaccaacgtgtacgccgacagcttcgtgatcagaggcaacgaggtgagccaaatcgcccctgggcagaccggcaacatcgccgactacaactacaagctgcccgacgacttcaccggctgcgtgatcgcctggaacagcaacaagctggacagcaaacctagcggcaactacaactacctgtacagactgttcagaaagagcaagctgaagcccttcgagagagacatcagcaccgagatctaccaagccggcaacaagccctgcaacggcgtggccggccccaactgctacagccccctgcagagctacggcttcagacccacctacggcgtgggccatcagccctacagagtggtcgtgctgagcttcgagctgctgcacgcccccgccaccgtgtgcggccccaagaagagcaccaacctggtgaagaacaagtgcgtgaacttcaacttcaacggcctcaccggcaccggcgtgctgaccgagagcaacaagaagttcctgccctttcagcagttcggcagagacatcgccgacaccaccgacgccgtgagagaccctcagaccctggagatcctggacatcaccccctgtagcttcggcggcgtgagcgtgatcacccccggcaccaacacaagcaaccaagtggccgtgctgtaccaaggcgtgaactgcaccgaggtgcccgtggccatccacgccgatcagctgacccccacctggagagtctactccaccggcagcaacgtgtttcagacaagagccggctgcctgatcggcgccgagtacgtgaacaacagctacgagtgcgacatccccatcggcgccggcatctgcgctagctatcagacacagaccaagagccacggcagcgctagcagcgtggctagccaaagcatcatcgcctacaccatgagcctgggcgccgagaacagcgtggcctacagcaacaacagcatcgccatccccaccaacttcaccatcagcgtgaccaccgagatcctgcccgtcagcatgaccaagacaagcgtggactgcaccatgtacatctgcggcgacagcaccgagtgcagcaacctgctcctgcagtacggcagcttctgcacacagctgaagagagccctgaccggcatcgccgtggagcaagacaagaacacccaagaggtgttcgcccaagtgaagcagatctacaagaccccccccatcaagtacttcggcggcttcaacttcagccaaatcctccccgacccctccaaacctagcaagagaagcttcatcgaggacctgctgttcaacaaggtgaccctggccgacgccggcttcatcaagcagtacggcgactgcctgggcgatatcgccgctagagacctgatctgcgctcagaagttcaatggcctgaccgtgctgccccccctgctgaccgacgagatgatcgctcagtatacaagcgctctgctcgctggcaccattacaagcgggtggaccttcggcgctggcgctgccctgcagatccccttcgccatgcagatggcctacagattcaacggcatcggcgtgacacagaacgtgctgtacgagaatcagaagctgatcgccaatcagttcaacagcgccatcggcaagatccaagacagcctgagcagcaccgctagcgccctgggcaagctgcaagacgtggtgaaccacaacgcccaagccctgaacaccctggtgaagcagctgagcagcaagttcggcgccatcagcagcgtgctcaacgacatcctgagcagactggacccccccgaggccgaggtgcagatcgatagactgatcaccggcagactgcagagcctgcagacctacgtgacacagcagctgatcagagccgccgagatcagagctagcgccaacctggccgccaccaagatgagcgagtgcgtgctggggcagagcaagagagtggacttctgcggcaagggctaccacctgatgagcttccctcagagcgccccccacggcgtggtgttcctgcacgtgacctacgtgcccgcccaagagaagaacttcaccacagcccccgccatctgccacgacggcaaggcccacttccctagagagggcgtgttcgtgagcaacggcacccactggttcgtgacacagagaaacttctacgagcctcagatcatcaccaccgacaacaccttcgtgagcggcaactgcgacgtggtgatcggcatcgtgaataataccgtgtacgaccccctgcagcccgagctggacagcttcaaggaggagctggacaagtatttcaagaaccatacaagccccgacgtggacctgggcgacatcagcggcatcaacgctagcgtggtgaacattcagaaggaaatcgacagactcaacgaggtggccaagaacctgaacgagagcctgatcgacctgcaagagctgggcaagtacgagcagtacatcaagtggccctggtacatctggctgggcttcatcgccggcctgatcgccatcgtgatggtgaccatcatgctgtgctgcatgacaagctgctgcagctgcctgaagggctgttgcagctgcggcagctgctgcaagttcgacgaggacgacagcgagcccgtgctgaagggcgtgaagctgcactacacctga

SEQ ID NO: 45 - DNA, 3810 bp, synthetic construct
  source 1..3810: mol_type = other DNA
atgttcgtgttcctggtgctgctgcccctggtgagcagccaatgcgtgaacctgatcacaagaacacagagctacaccaacagcttcacaagaggcgtgtactaccccgacaaggtgttcagaagcagcgtgctgcactccacccaagacctgtttctgccctttttcagcaacgtgacctggttccacgccatccacgtgagcggcaccaacggcaccaagagattcgacaaccccgccctgcccttcaacgacggcgtgtacttcgctagcaccgagaagagcaacatcatcagaggctggatcttcggcaccaccctggacagcaaaacacagagcctgctgatcgtgaacaatgccaccaacgtggtgatcaaggtgtgcgagtttcagttctgcaacgaccccttcctggacgtgtatcagaagaacaacaagagctggatggagagcgagttcagagtgtacagctccgccaacaactgcaccttcgagtacgtgagccaacccttcctgatggacctggagggcaaggagggcaacttcaagaacctccgggagttcgtgttcaagaacatcgacggctacttcaagatctacagcaagcacacccccatcaacctggagagagacctgccccaaggcttcagcgccctggagcccctggtggacctgcccatcggcatcaacatcacaagatttcagaccctgctggctctgcacagaagctatctcacccccggcgggagcagcagcggctggaccgccggggctgctgcctactacgtgggctacctgcagcctagaaccttcctgctgaagtacaacgagaacggcaccattaccgatgccgtggactgtgccctggaccccctgagcgagaccaagtgcaccctgaagagcttcaccgtggagaagggcatctatcagacaagcaacttcagagtgcagcccaccgagagcatcgtgagattccccaacatcaccaacctgtgccccttccacgaggtgttcaacgccaccaccttcgctagcgtgtacgcctggaaccggaagagaatcagcaactgcgtggccgactacagcgtgatctacaacttcgcccccttcttcgccttcaaatgctacggcgtgagccccaccaagctgaacgacctgtgcttcaccaacgtgtacgccgacagcttcgtgatcagaggcaacgaggtgagccaaatcgcccctgggcagaccggcaacatcgccgactacaactacaagctgcccgacgacttcaccggctgcgtgatcgcctggaactccaacaagctggacagcaagcctagcggcaactacaactacctgtacagactgttcagaaagagcaagctgaagcccttcgagagagacatcagcaccgagatctaccaagccggcaacaagccctgcaacggcgtggccggccccaactgctacagccccctgcagagctacggcttcagacccacctacggcgtgggccatcagccctacagagtggtcgtgctgagcttcgagctgctgcacgctagcgccaccgtgtgcggccccaagaagagcaccaacctggtgaagaacaagtgcgtgaacttcaacttcaacggcctgaccggcaccggcgtgctgaccgagagcaacaagaagttcctgccctttcagcagttcggcagagacatcgccgacaccaccgacgccgtgagagaccctcagaccctggagatcctggacatcaccccttgcagcttcgggggcgtgagcgtgatcacccccggcaccaacacaagcaaccaagtggccgtgctgtaccaaggcgtgaactgcaccgaggtgcccgtggccatccacgccgatcagctgacccccacctggcgggtgtatagcaccggcagcaacgtgtttcagacaagagccggctgcctgatcggcgccgagtacgtgaacaacagctacgagtgcgacatccccatcggcgccggcatctgcgctagctatcagacacagaccaagagccacggcagcgctagcagcgtggctagccaaagcatcatcgcctacaccatgagcctgggcgccgagaacagcgtggcctacagcaacaacagcatcgccatccccaccaacttcaccatcagcgtgaccaccgaaatcctgcccgtgtccatgaccaagacaagcgtggactgcaccatgtacatctgcggcgacagcaccgagtgcagcaacctgctcctgcagtacggcagcttctgcacacagctgaagagagccctgaccggcatcgccgtggagcaagacaagaacacccaagaggtgttcgcccaagtgaagcagatctacaagaccccccccatcaagtacttcggcggcttcaacttcagccaaatcctgcccgaccctagcaagcctagcaagagaagccccatcgaggacctgctgttcaacaaggtgaccctggccgacgccggcttcatcaagcagtacggcgactgcctcggcgacattgctgctagagacctgatctgcgctcagaagttcaacggcctcacagtcctcccccccctgctgaccgacgagatgattgctcagtacacaagcgccctgctggccggcaccattacaagcgggtggacctttggcgctggccctgccctgcagatccccttccccatgcagatggcctacagattcaacggcatcggcgtgacacagaacgtgctgtacgagaatcagaagctgatcgccaatcagttcaacagcgccatcggcaagatccaagacagcctgagcagcacccctagcgccctgggcaagctgcaagacgtggtgaaccacaacgcccaagccctgaacaccctggtgaagcagctgagcagcaagttcggcgccatctcctccgtgctgaatgacatcctgagcagactggacccccccgaggccgaggtgcagattgacagactgatcaccggcagactgcagagcctgcagacctacgtgacacagcagctgatcagagccgccgagatcagagctagcgccaacctggccgccaccaagatgagcgagtgcgtgctggggcagagcaagagagtggacttctgcggcaagggctaccacctgatgagcttccctcagagcgccccccacggcgtggtgttcctgcacgtgacctacgtgcccgcccaagagaagaacttcaccaccgcccccgccatctgccacgacggcaaggcccacttccctagagagggcgtgttcgtgagcaacggcacccactggttcgtgacacagagaaacttctacgagcctcagatcatcaccaccgacaacaccttcgtgagcggcaactgcgacgtggtgatcggcatcgtgaacaacacagtgtacgaccccctgcagcccgagctggacagcttcaaggaggagctggacaagtactttaaaaaccacacaagccccgacgtggacctcggcgacatctccggcatcaacgctagcgtggtgaacattcagaaggagatcgatagactgaacgaggtggccaagaacctgaacgagagcctgatcgacctgcaagagctgggcaagtacgagcagtacatcaagtggccctggtacatctggctgggcttcatcgccggcctgatcgccatcgtgatggtgaccatcatgctgtgctgcatgacaagctgctgctcctgcctgaaggggtgctgcagctgcggcagctgctgcaagttcgacgaggacgacagcgagcccgtgctgaagggcgtgaagctgcactacacctga

SEQ ID NO: 46 - protein, 323 aa, synthetic construct
VQPTESIVRFPNVTNLCPFHEVFNATRFASVYAWNRTRISNCVADYSVLYNFAPFFAFKCYGVSPTKLNDLCFTNVYADSFVIKGNEVSQIAPGQTGNIADYNYKLPDDFTGCVIAWNSNKLDSKHSGNYDYWYRSFRKSKLKPFERDISTEIYQAGNKPCKGKGPNCYFPLQSYGFRPTYGVGHQPYRVVVLSFELLHAPATVCGPKKSTNLVKNKSVNFNFNGLYENQKLIANQFNSAIGKIQDSLSSTASALGKLQDVVNQNAQALNTLVKQLKNHTSPDVDLGDISGINASVVNIQKEIDRLNEVAKNLNESLIDLQEL

SEQ ID NO: 47 - protein, 491 aa, synthetic construct
MLLVNQSHQGFNKEHTSKMVSAIVLYVLLAAAAHSAFAADSIHIKDSDDLKNRLAEAGDKLVVIDFMATWCGPCKMIGPKLDEMANEMSDSIVVLKVDVDECEDIATEYNINSMPTFVFVKNSKKIEEFSGANVDKLRNTIIKLKLAGSGSGHMHHHHHHSSGDDDDKVQPTESIVRFPNVTNLCPFHEVFNATRFASVYAWNRTRISNCVADYSVLYNFAPFFAFKCYGVSPTKLNDLCFTNVYADSFVIKGNEVSQIAPGQTGNIADYNYKLPDDFTGCVIAWNSNKLDSKHSGNYDYWYRSFRKSKLKPFERDISTEIYQAGNKPCKGKGPNCYFPLQSYGFRPTYGVGHQPYRVVVLSFELLHAPATVCGPKKSTNLVKNKSVNFNFNGLYENQKLIANQFNSAIGKIQDSLSSTASALGKLQDVVNQNAQALNTLVKQLKNHTSPDVDLGDISGINASVVNIQKEIDRLNEVAKNLNESLIDLQEL

SEQ ID NO: 48 - DNA, 1476 bp, synthetic construct
  source 1..1476: mol_type = other DNA
atgctgctggtgaaccagagccaccagggtttcaacaaggaacacactagcaagatggtgtctgctatcgtcctctacgtgctgctcgccgccgctgctcactcagctttcgccgctgactctatccacatcaaggactccgacgacctcaagaaccgtttggccgaagccggcgacaagctggtcgttatcgacttcatggctacctggtgtggcccttgcaagatgatcggacctaagctggacgaaatggctaacgagatgagcgacagcatcgtcgttctgaaggtggacgtcgacgaatgtgaggacatcgccactgagtacaacatcaacagcatgcctaccttcgttttcgtgaagaactctaagaagatcgaggagttctctggtgccaacgtggacaagctccgtaacaccatcatcaagctcaagctggccggcagcggtagcggtcacatgcaccaccaccaccaccattcaagcggcgacgacgacgacaaggtgcagccaaccgaatcaatcgtccgcttcccaaacgtcactaacctgtgcccattccacgaggtgttcaacgccacccgtttcgcctctgtctacgcttggaaccgcacgcgcatctccaactgtgtcgccgactacagcgtgctgtacaacttcgctcctttcttcgcattcaagtgttacggagtgtcccctaccaagctcaacgatttgtgcttcacaaacgtgtacgctgacagcttcgtgatcaagggtaacgaggtttctcaaatcgcccctggtcagacaggtaacatcgctgactacaactacaagctcccagacgacttcactggctgtgttatcgcttggaactcaaacaagctggactctaagcattctggtaactacgactactggtaccgttcgttccgcaagagcaagctcaagccattcgaacgtgacatcagcacagagatctaccaagccggtaacaagccctgcaagggcaagggacctaactgctacttccccctccagtcctacggattccgcccaacctacggcgtgggtcaccagccataccgcgtggttgtgctgagcttcgaactgctgcacgcccccgctaccgtgtgtggccctaagaagagcactaacctcgttaagaacaagtccgtgaacttcaacttcaacggtctctacgaaaaccagaagctgatcgctaaccagttcaactccgccatcggcaagatccaggactccctgtcctccacagcttccgctctgggcaagctgcaggacgttgtgaaccaaaacgctcaggccctgaacacactggtgaagcaactgaagaaccacaccagccccgacgttgacctgggtgacatcagcggtatcaacgctagcgtggtgaacatccagaaggagatcgacaggctgaacgaagtggctaagaacttgaacgagagcctcatcgacctgcaggaactgtaa

SEQ ID NO: 49 - DNA, 20 bp, synthetic construct
  source 1..20: mol_type = other DNA
gaccccaaaatcagcgaaat

SEQ ID NO: 50 - DNA, 24 bp, synthetic construct
  source 1..24: mol_type = other DNA
tctggttactgccagttgaatctg

SEQ ID NO: 51 - DNA, 24 bp, synthetic construct
  source 1..24: mol_type = other DNA
acngccgcattacgttggtggacc